European Patent Application EP 4 414 381 A1, published August 14, 2024. Title: IL10 MONOMER FUSION PROTEIN AND USE THEREOF. Applicant: Guangdong Fapon Biopharma Inc. The sequence listing filed with the application follows.

SEQUENCE LISTING (23 sequences)

SEQ ID NO: 1 - protein, 160 aa, synthetic construct
SPGQGTQSENSCTHFPGNLPNMLRDLRDAFSRVKTFFQMKDQLDNLLLKESLLEDFKGYLGCQALSEMIQFYLEEVMPQAENQDPDIKAHVNSLGENLKTLRLRLRRCHRFLPCENKSKAVEQVKNAFNKLQEKGIYKAMSEFDIFINYIEAYMTMKIRN

SEQ ID NO: 2 - protein, 164 aa, synthetic construct
GQGTQSENSCTHFPGNLPNMLRDLRDAFSRVKTFFQMKDQLDNLLLKESLLEDFKGYLGCQALSEMIQFYLEEVMPQAENQDPDIKAHVNSLGENLKTLRLRLRRCHRFLPCENGGGSGGKSKAVEQVKNAFNKLQEKGIYKAMSEFDIFINYIEAYMTMKIRN

SEQ ID NO: 3 - protein, 451 aa, synthetic construct
QVQLKESGPGLVQPSQTLSLTCTVSGFSLTSYNVHWVRQPPGKGLEWMGGMRYNEDTSYNSALKSRLSISRDTSKNQVFLKMNSLQTDDTGTYYCTRDAVYGGYGGWFAYWGQGTLVTVSSASTKGPSVFPLAPSSKSTSGGTAALGCLVKDYFPEPVTVSWNSGALTSGVHTFPAVLQSSGLYSLSSVVTVPSSSLGTQTYICNVNHKPSNTKVDKRVEPKSCDKTHTCPPCPAPEAAGGPSVFLFPPKPKDTLMISRTPEVTCVVVDVSHEDPEVKFNWYVDGVEVHNAKTKPREEQYNSTYRVVSVLTVLHQDWLNGKEYKCKVSNKALPAPIEKTISKAKGQPREPQVYTLPPSREEMTKNQVSLTCLVKGFYPSDIAVEWESNGQPENNYKTTPPVLDSDGSFFLYSKLTVDKSRWQQGNVFSCSVMHEALHNHYTQKSLSLSPGK

SEQ ID NO: 4 - protein, 631 aa, synthetic construct
QVQLKESGPGLVQPSQTLSLTCTVSGFSLTSYNVHWVRQPPGKGLEWMGGMRYNEDTSYNSALKSRLSISRDTSKNQVFLKMNSLQTDDTGTYYCTRDAVYGGYGGWFAYWGQGTLVTVSSGSGSGSGSGQGTQSENSCTHFPGNLPNMLRDLRDAFSRVKTFFQMKDQLDNLLLKESLLEDFKGYLGCQALSEMIQFYLEEVMPQAENQDPDIKAHVNSLGENLKTLRLRLRRCHRFLPCENGGGSGGKSKAVEQVKNAFNKLQEKGIYKAMSEFDIFINYIEAYMTMKIRNGSGSGSGSASTKGPSVFPLAPSSKSTSGGTAALGCLVKDYFPEPVTVSWNSGALTSGVHTFPAVLQSSGLYSLSSVVTVPSSSLGTQTYICNVNHKPSNTKVDKRVEPKSCDKTHTCPPCPAPEAAGGPSVFLFPPKPKDTLMISRTPEVTCVVVDVSHEDPEVKFNWYVDGVEVHNAKTKPREEQYNSTYRVVSVLTVLHQDWLNGKEYKCKVSNKALPAPIEKTISKAKGQPREPQVYTLPPSREEMTKNQVSLTCLVKGFYPSDIAVEWESNGQPENNYKTTPPVLDSDGSFFLYSKLTVDKSRWQQGNVFSCSVMHEALHNHYTQKSLSLSPGK

SEQ ID NO: 5 - protein, 396 aa, synthetic construct
DTVLTQSPALAVSLGQRVTISCKASETVSSSMYSYIHWYQQKPGQQPKLLIYRASNLESGVPARFSGSGSGTDFTLTIDPVEADDVATYFCQQSWNPWTFGGGTKLELKRGSGSGSGSGQGTQSENSCTHFPGNLPNMLRDLRDAFSRVKTFFQMKDQLDNLLLKESLLEDFKGYLGCQALSEMIQFYLEEVMPQAENQDPDIKAHVNSLGENLKTLRLRLRRCHRFLPCENGGGSGGKSKAVEQVKNAFNKLQEKGIYKAMSEFDIFINYIEAYMTMKIRNGSGSGSGSTVAAPSVFIFPPSDEQLKSGTASVVCLLNNFYPREAKVQWKVDNALQSGNSQESVTEQDSKDSTYSLSSTLTLSKADYEKHKVYACEVTHQGLSSPVTKSFNRGEC

SEQ ID NO: 6 - protein, 216 aa, synthetic construct
DTVLTQSPALAVSLGQRVTISCKASETVSSSMYSYIHWYQQKPGQQPKLLIYRASNLESGVPARFSGSGSGTDFTLTIDPVEADDVATYFCQQSWNPWTFGGGTKLELKRTVAAPSVFIFPPSDEQLKSGTASVVCLLNNFYPREAKVQWKVDNALQSGNSQESVTEQDSKDSTYSLSSTLTLSKADYEKHKVYACEVTHQGLSSPVTKSFNRGEC

SEQ ID NO: 7 - protein, 631 aa, synthetic construct
QVQLKESGPGLVQPSQTLSLTCTVSGFSLTSYNVHWVRQPPGKGLEWMGGMRYNEDTSYNSALKSRLSISRDTSKNQVFLKMNSLQTDDTGTYYCTRDAVYGGYGGWFAYWGQGTLVTVSSASTKGPSVFPLAPSSKSTSGGTAALGCLVKDYFPEPVTVSWNSGALTSGVHTFPAVLQSSGLYSLSSVVTVPSSSLGTQTYICNVNHKPSNTKVDKRVEPKSCDKTHTCPPCPAPEAAGGPSVFLFPPKPKDTLMISRTPEVTCVVVDVSHEDPEVKFNWYVDGVEVHNAKTKPREEQYNSTYRVVSVLTVLHQDWLNGKEYKCKVSNKALPAPIEKTISKAKGSGSGSGSGQGTQSENSCTHFPGNLPNMLRDLRDAFSRVKTFFQMKDQLDNLLLKESLLEDFKGYLGCQALSEMIQFYLEEVMPQAENQDPDIKAHVNSLGENLKTLRLRLRRCHRFLPCENGGGSGGKSKAVEQVKNAFNKLQEKGIYKAMSEFDIFINYIEAYMTMKIRNGSGSGSGSGQPREPQVYTLPPSREEMTKNQVSLTCLVKGFYPSDIAVEWESNGQPENNYKTTPPVLDSDGSFFLYSKLTVDKSRWQQGNVFSCSVMHEALHNHYTQKSLSLSPGK

SEQ ID NO: 8 - protein, 401 aa, synthetic construct
GQGTQSENSCTHFPGNLPNMLRDLRDAFSRVKTFFQMKDQLDNLLLKESLLEDFKGYLGCQALSEMIQFYLEEVMPQAENQDPDIKAHVNSLGENLKTLRLRLRRCHRFLPCENGGGSGGKSKAVEQVKNAFNKLQEKGIYKAMSEFDIFINYIEAYMTMKIRNGGGGSGGGGSGGGGSGGGGSGDTVLTQSPALAVSLGQRVTISCKASETVSSSMYSYIHWYQQKPGQQPKLLIYRASNLESGVPARFSGSGSGTDFTLTIDPVEADDVATYFCQQSWNPWTFGGGTKLELKRTVAAPSVFIFPPSDEQLKSGTASVVCLLNNFYPREAKVQWKVDNALQSGNSQESVTEQDSKDSTYSLSSTLTLSKADYEKHKVYACEVTHQGLSSPVTKSFNRGEC

SEQ ID NO: 9 - protein, 401 aa, synthetic construct
DTVLTQSPALAVSLGQRVTISCKASETVSSSMYSYIHWYQQKPGQQPKLLIYRASNLESGVPARFSGSGSGTDFTLTIDPVEADDVATYFCQQSWNPWTFGGGTKLELKRTVAAPSVFIFPPSDEQLKSGTASVVCLLNNFYPREAKVQWKVDNALQSGNSQESVTEQDSKDSTYSLSSTLTLSKADYEKHKVYACEVTHQGLSSPVTKSFNRGECGGGGSGGGGSGGGGSGGGGSGGQGTQSENSCTHFPGNLPNMLRDLRDAFSRVKTFFQMKDQLDNLLLKESLLEDFKGYLGCQALSEMIQFYLEEVMPQAENQDPDIKAHVNSLGENLKTLRLRLRRCHRFLPCENGGGSGGKSKAVEQVKNAFNKLQEKGIYKAMSEFDIFINYIEAYMTMKIRN

SEQ ID NO: 10 - protein, 636 aa, synthetic construct
GQGTQSENSCTHFPGNLPNMLRDLRDAFSRVKTFFQMKDQLDNLLLKESLLEDFKGYLGCQALSEMIQFYLEEVMPQAENQDPDIKAHVNSLGENLKTLRLRLRRCHRFLPCENGGGSGGKSKAVEQVKNAFNKLQEKGIYKAMSEFDIFINYIEAYMTMKIRNGGGGSGGGGSGGGGSGGGGSGQVQLKESGPGLVQPSQTLSLTCTVSGFSLTSYNVHWVRQPPGKGLEWMGGMRYNEDTSYNSALKSRLSISRDTSKNQVFLKMNSLQTDDTGTYYCTRDAVYGGYGGWFAYWGQGTLVTVSSASTKGPSVFPLAPSSKSTSGGTAALGCLVKDYFPEPVTVSWNSGALTSGVHTFPAVLQSSGLYSLSSVVTVPSSSLGTQTYICNVNHKPSNTKVDKRVEPKSCDKTHTCPPCPAPEAAGGPSVFLFPPKPKDTLMISRTPEVTCVVVDVSHEDPEVKFNWYVDGVEVHNAKTKPREEQYNSTYRVVSVLTVLHQDWLNGKEYKCKVSNKALPAPIEKTISKAKGQPREPQVYTLPPSREEMTKNQVSLTCLVKGFYPSDIAVEWESNGQPENNYKTTPPVLDSDGSFFLYSKLTVDKSRWQQGNVFSCSVMHEALHNHYTQKSLSLSPGK

SEQ ID NO: 11 - protein, 636 aa, synthetic construct; identical to SEQ ID NO: 10

SEQ ID NO: 12 - protein, 8 aa, synthetic construct
GSGSGSGS

SEQ ID NO: 13 - protein, 445 aa, synthetic construct
QVQLKESGPGLVQPSQTLSLTCTVSGFSLTSYNVHWVRQPPGKGLEWMGGMRYNEDTSYNSALKSRLSISRDTSKNQVFLKMNSLQTDDTGTYYCTRDAVYGGYGGWFAYWGQGTLVTVSSAKTTPPSVYPLAPGSAAQTNSMVTLGCLVKGYFPEPVTVTWNSGSLSSGVHTFPAVLQSDLYTLSSSVTVPSSTWPSQTVTCNVAHPASSTKVDKKIVPRDCGCKPCICTVPEVSSVFIFPPKPKDVLTITLTPKVTCVVVDISKDDPEVQFSWFVDDVEVHTAQTKPREEQFNSTFRSVSELPIMHQDWLNGKEFKCRVNSAAFPAPIEKTISKTKGRPKAPQVYTIPPPKEQMAKDKVSLTCMITNFFPEDITVEWQWNGQPAENYKNTQPIMDTDGSYFVYSKLNVQKSNWEAGNTFTCSVLHEGLHNHHTEKSLSHSPGK

SEQ ID NO: 14 - protein, 216 aa, synthetic construct
DTVLTQSPALAVSLGQRVTISCKASETVSSSMYSYIHWYQQKPGQQPKLLIYRASNLESGVPARFSGSGSGTDFTLTIDPVEADDVATYFCQQSWNPWTFGGGTKLELKRADAAPTVSIFPPSSEQLTSGGASVVCFLNNFYPKDINVKWKIDGSERQNGVLNSWTDQDSKDSTYSMSSTLTLTKDEYERHNSYTCEATHKTSTSPIVKSFNRNEC

SEQ ID NO: 15 - protein, 400 aa, synthetic construct
GQGTQSENSCTHFPGNLPNMLRDLRDAFSRVKTFFQMKDQLDNLLLKESLLEDFKGYLGCQALSEMIQFYLEEVMPQAENQDPDIKAHVNSLGENLKTLRLRLRRCHRFLPCENKSKAVEQVKNAFNKLQEKGIYKAMSEFDIFINYIEAYMTMKIRNGGGSGSGSGSEPKSSDKTHTCPPCPAPELAGAPSVFLFPPKPKDTLMISRTPEVTCVVVDVSHEDPEVKFNWYVDGVEVHNAKTKPREEQYNSTYRVVSVLTVLHQDWLNGKEYKCKVSNKQLPAPIEKTISKAKGQPREPQVYTLPPSRDELTKNQVSLTCLVKGFYPSDIAVEWESNGQPENNYKTTPPVLDSDGSFFLYSKLTVDKSRWQQGNVFSCSVMHEALHNHYTQKSLSLSPGK

SEQ ID NO: 16 - protein, 449 aa, synthetic construct
QVQLVESGGGVVQPGRSLRLSCAASGFTFSSYGMHWVRQAPGKGLEWVAAIWYDGSNKYYTDSVKGRFTISRDNSKNTLYLQMNSLRAEDTAVYYCARDLRGVMYFDLWGRGTLVTVSSASTKGPSVFPLAPSSKSTSGGTAALGCLVKDYFPEPVTVSWNSGALTSGVHTFPAVLQSSGLYSLSSVVTVPSSSLGTQTYICNVNHKPSNTKVDKRVEPKSCDKTHTCPPCPAPEAAGGPSVFLFPPKPKDTLMISRTPEVTCVVVDVSHEDPEVKFNWYVDGVEVHNAKTKPREEQYNSTYRVVSVLTVLHQDWLNGKEYKCKVSNKALPAPIEKTISKAKGQPREPQVYTLPPSREEMTKNQVSLTCLVKGFYPSDIAVEWESNGQPENNYKTTPPVLDSDGSFFLYSKLTVDKSRWQQGNVFSCSVMHEALHNHYTQKSLSLSPGK

SEQ ID NO: 17 - protein, 214 aa, synthetic construct
EIVLTQSPATLSLSPGERATLSCRASQSVSRYLAWYQQKPGQAPRLLIYDASNRATGIPARFSGSGSGTDFTLTISSLEPEDFAVYYCQLRNNWPLTFGGGTKVEIKRTVAAPSVFIFPPSDEQLKSGTASVVCLLNNFYPREAKVQWKVDNALQSGNSQESVTEQDSKDSTYSLSSTLTLSKADYEKHKVYACEVTHQGLSSPVTKSFNRGEC

SEQ ID NO: 18 - protein, 407 aa, synthetic construct
DKTHTCPPCPAPEAEGGPSVFLFPPKPKDTLMISRTPEVTCVVVDVSHEDPEVKFNWYVDGVEVHNAKTKPREEQYNSTYRVVSVLTVLHQDWLNGKEYKCKVSNKALPAPIEKTISKAKGQPREPQVYTLPPSREEMTKNQVSLTCLVKGFYPSDIAVEWESNGQPENNYKTTPPVLDSDGSFFLYSKLTVDKSRWQQGNVFSCSVMHEALHNHYTQKSLSLSPGKGGGGSGGGGSGGGGSGGGGSSPGQGTQSENSCTHFPGNLPNMLRDLRDAFSRVKTFFQMKDQLDNLLLKESLLEDFKGYLGCQALSEMIQFYLEEVMPQAENQDPDIKAHVNSLGENLKTLRLRLRRCHRFLPCENKSKAVEQVKNAFNKLQEKGIYKAMSEFDIFINYIEAYMTMKIRN

SEQ ID NO: 19 - protein, 451 aa, synthetic construct; identical to SEQ ID NO: 3

SEQ ID NO: 20 - protein, 216 aa, synthetic construct; identical to SEQ ID NO: 6

SEQ ID NO: 21 - protein, 6 aa, synthetic construct
GGGSGG

SEQ ID NO: 22 - protein, 21 aa, synthetic construct
GGGGSGGGGSGGGGSGGGGSG

SEQ ID NO: 23 - protein, 626 aa, synthetic construct
QVQLKESGPGLVQPSQTLSLTCTVSGFSLTSYNVHWVRQPPGKGLEWMGGMRYNEDTSYNSALKSRLSISRDTSKNQVFLKMNSLQTDDTGTYYCTRDAVYGGYGGWFAYWGQGTLVTVSSAKTTPPSVYPLAPGSAAQTNSMVTLGCLVKGYFPEPVTVTWNSGSLSSGVHTFPAVLQSDLYTLSSSVTVPSSTWPSQTVTCNVAHPASSTKVDKKIVPRDCGCKPCICTVPEVSSVFIFPPKPKDVLTITLTPKVTCVVVAISKDDPEVQFSWFVDDVEVHTAQTKPREEQFNSTFRSVSELPIMHQDWLNGKEFKCRVNSAAFPAPIEKTISKTKGRPKAPQVYTIPPPKEQMAKDKVSLTCMITNFFPEDITVEWQWNGQPAENYKNTQPIMDTDGSYFVYSKLNVQKSNWEAGNTFTCSVLHEGLHNHHTEKSLSHSPGAGGGGSGGGGSGGGGSGGGGSGSPGQGTQSENSCTHFPGNLPNMLRDLRDAFSRVKTFFQMKDQLDNLLLKESLLEDFKGYLGCQALSEMIQFYLEEVMPQAENQDPDIKAHVNSLGENLKTLRLRLRRCHRFLPCENKSKAVEQVKNAFNKLQEKGIYKAMSEFDIFINYIEAYMTMKIRN